European Patent Application EP 4 299 744 A1, published January 3, 2024. Title: Oligonucleotide for inducing N-exon skipping in processing of REST pre-mRNA. Applicant: Osaka University. The sequence listing filed with the application follows.

SEQUENCE LISTING (67 sequences)

SEQ ID NO: 1 - RNA, 50 nt, Homo sapiens
ugggguauggauaccauuugguaauauuuacuagagugugaucuagaugg

SEQ ID NO: 2 - RNA, 138 nt, Homo sapiens
uuuucauaaaugucaauuuccguuuuucuacuaugcauuccauuggaccagugggguauggauaccauuugguaauauuuacuagagugugaucuagauggguauguauucagguagaauguauuacucuuaugccuu

SEQ ID NO: 3 - DNA, 18 bp, Artificial Sequence
  [+1/+18]
aatggtatccatacccca

SEQ ID NO: 4 - DNA, 18 bp, Artificial Sequence
  [+5/+22]
accaaatggtatccatac

SEQ ID NO: 5 - DNA, 18 bp, Artificial Sequence
  [+13/+30]
taaatattaccaaatggt

SEQ ID NO: 6 - DNA, 18 bp, Artificial Sequence
  [+15/+32]
agtaaatattaccaaatg

SEQ ID NO: 7 - DNA, 18 bp, Artificial Sequence
  [+19/+36]
ctctagtaaatattacca

SEQ ID NO: 8 - DNA, 18 bp, Artificial Sequence
  [+23/+40]
cacactctagtaaatatt

SEQ ID NO: 9 - DNA, 18 bp, Artificial Sequence
  [+27/+44]
agatcacactctagtaaa

SEQ ID NO: 10 - DNA, 18 bp, Artificial Sequence
  [+31/+48]
atctagatcacactctag

SEQ ID NO: 11 - DNA, 18 bp, Artificial Sequence
  [+35/-2(3')]
acccatctagatcacact

SEQ ID NO: 12 - DNA, 18 bp, Artificial Sequence
  AmNA[-44/-27]
  modified_base (1)..(1): a = AmNA_a
  modified_base (2)..(18): phosphorotioated
  modified_base (3)..(3): a = AmNA_a
  modified_base (5)..(5): g = AmNA_g
  modified_base (7)..(7): a = AmNA_a
  modified_base (9)..(9): a = AmNA_a
  modified_base (11)..(11): t = AmNA_t
  modified_base (13)..(13): a = AmNA_a
  modified_base (15)..(15): a = AmNA_a
  modified_base (17)..(17): t = AmNA_t
aaacggaaattgacattt

SEQ ID NO: 13 - DNA, 18 bp, Artificial Sequence
  AmNA[-32/-15]
  modified_base (1)..(1): t = AmNA_t
  modified_base (2)..(18): phosphorotioated
  modified_base (3)..(3): c = AmNA_c
  modified_base (3)..(3): m5c
  modified_base (5)..(5): t = AmNA_t
  modified_base (7)..(7): g = AmNA_g
  modified_base (9)..(9): a = AmNA_a
  modified_base (11)..(11): a = AmNA_a
  modified_base (13)..(13): a = AmNA_a
  modified_base (15)..(15): a = AmNA_a
  modified_base (17)..(17): g = AmNA_g
tgcatagtagaaaaacgg

SEQ ID NO: 14 - DNA, 18 bp, Artificial Sequence
  AmNA[-24/-7]
  modified_base (1)..(1): c = AmNA_c
  modified_base (1)..(1): m5c
  modified_base (2)..(18): phosphorotioated
  modified_base (3)..(3): a = AmNA_a
  modified_base (5)..(5): g = AmNA_g
  modified_base (7)..(7): a = AmNA_a
  modified_base (9)..(9): t = AmNA_t
  modified_base (11)..(11): m5c
  modified_base (11)..(11): c = AmNA_c
  modified_base (13)..(13): t = AmNA_t
  modified_base (15)..(15): g = AmNA_g
  modified_base (17)..(17): a = AmNA_a
caatggaatgcatagtag

SEQ ID NO: 15 - DNA, 18 bp, Artificial Sequence
  AmNA[-20/-3]
  modified_base (1)..(1): g = AmNA_g
  modified_base (2)..(18): phosphorotioated
  modified_base (2)..(18): phosphorotioated
  modified_base (3)..(3): t = AmNA_t
  modified_base (5)..(5): c = AmNA_c
  modified_base (5)..(5): m5c
  modified_base (7)..(7): a = AmNA_a
  modified_base (9)..(9): g = AmNA_g
  modified_base (11)..(11): a = AmNA_a
  modified_base (13)..(13): t = AmNA_t
  modified_base (15)..(15): c = AmNA_c
  modified_base (17)..(17): t = AmNA_t
ggtccaatggaatgcata

SEQ ID NO: 16 - DNA, 18 bp, Artificial Sequence
  AmNA[-18/-1]
  modified_base (1)..(1): c = AmNA_c
  modified_base (1)..(1): m5c
  modified_base (2)..(18): phosphorotioated
  modified_base (3)..(3): g = AmNA_g
  modified_base (5)..(5): t = AmNA_t
  modified_base (7)..(7): c = AmNA_c
  modified_base (7)..(7): m5c
  modified_base (9)..(9): a = AmNA_a
  modified_base (11)..(11): g = AmNA_g
  modified_base (13)..(13): a = AmNA_a
  modified_base (15)..(15): t = AmNA_t
  modified_base (17)..(17): c = AmNA_c
  modified_base (17)..(17): m5c
ctggtccaatggaatgca

SEQ ID NO: 17 - DNA, 18 bp, Artificial Sequence
  AmNA[-8/+10]
  modified_base (1)..(1): c = AmNA_c
  modified_base (1)..(1): m5c
  modified_base (2)..(18): phosphorotioated
  modified_base (5)..(5): a = AmNA_a
  modified_base (7)..(7): c = AmNA_c
  modified_base (7)..(7): m5c
  modified_base (9)..(9): c = AmNA_c
  modified_base (9)..(9): m5c
  modified_base (11)..(11): c = AmNA_c
  modified_base (11)..(11): m5c
  modified_base (13)..(13): g = AmNA_g
  modified_base (15)..(15): t = AmNA_t
  modified_base (17)..(17): c = AmNA_c
  modified_base (17)..(17): m5c
ccataccccactggtcca

SEQ ID NO: 18 - DNA, 18 bp, Artificial Sequence
  AmNA[+1/+18]
  modified_base (1)..(1): a = AmNA_a
  modified_base (2)..(18): phosphorotioated
  modified_base (3)..(3): t = AmNA_t
  modified_base (5)..(5): g = AmNA_g
  modified_base (5)..(5): m5c
  modified_base (7)..(7): a = AmNA_a
  modified_base (9)..(9): c = AmNA_c
  modified_base (11)..(11): a = AmNA_a
  modified_base (15)..(15): c = AmNA_c
  modified_base (15)..(15): m5c
  modified_base (17)..(17): c = AmNA_c
  modified_base (17)..(17): m5c
aatggtatccatacccca

SEQ ID NO: 19 - DNA, 18 bp, Artificial Sequence
  AmNA[+5/+22]
  modified_base (1)..(1): a = AmNA_a
  modified_base (2)..(18): phosphorotioated
  modified_base (3)..(3): c = AmNA_c
  modified_base (3)..(3): m5c
  modified_base (5)..(5): a = AmNA_a
  modified_base (7)..(7): t = AmNA_t
  modified_base (9)..(9): g = AmNA_g
  modified_base (11)..(11): a = AmNA_a
  modified_base (13)..(13): c = AmNA_c
  modified_base (13)..(13): m5c
  modified_base (15)..(15): a = AmNA_a
  modified_base (17)..(17): a = AmNA_a
accaaatggtatccatac

SEQ ID NO: 20 - DNA, 18 bp, Artificial Sequence
  AmNA[+13/+30]
  modified_base (1)..(1): t = AmNA_t
  modified_base (2)..(18): phosphorotioated
  modified_base (3)..(3): a = AmNA_a
  modified_base (5)..(5): t = AmNA_t
  modified_base (7)..(7): t = AmNA_t
  modified_base (9)..(9): a = AmNA_a
  modified_base (11)..(11): c = AmNA_c
  modified_base (11)..(11): m5c
  modified_base (13)..(13): a = AmNA_a
  modified_base (15)..(15): t = AmNA_t
  modified_base (17)..(17): g = AmNA_g
taaatattaccaaatggt

SEQ ID NO: 21 - DNA, 18 bp, Artificial Sequence
  AmNA[+15/+32]
  modified_base (1)..(1): a = AmNA_a
  modified_base (2)..(18): phosphorotioated
  modified_base (3)..(3): t = AmNA_t
  modified_base (5)..(5): a = AmNA_a
  modified_base (7)..(7): t = AmNA_t
  modified_base (9)..(9): t = AmNA_t
  modified_base (11)..(11): a = AmNA_a
  modified_base (13)..(13): c = AmNA_c
  modified_base (13)..(13): m5c
  modified_base (15)..(15): a = AmNA_a
  modified_base (17)..(17): t = AmNA_t
agtaaatattaccaaatg

SEQ ID NO: 22 - DNA, 18 bp, Artificial Sequence
  AmNA[+19/+36]
  modified_base (1)..(1): c = AmNA_c
  modified_base (1)..(1): m5c
  modified_base (2)..(18): phosphorotioated
  modified_base (3)..(3): c = AmNA_c
  modified_base (3)..(3): m5c
  modified_base (5)..(5): a = AmNA_a
  modified_base (7)..(7): t = AmNA_t
  modified_base (9)..(9): a = AmNA_a
  modified_base (11)..(11): t = AmNA_t
  modified_base (13)..(13): t = AmNA_t
  modified_base (15)..(15): a = AmNA_a
  modified_base (17)..(17): c = AmNA_c
  modified_base (17)..(17): m5c
ctctagtaaatattacca

SEQ ID NO: 23 - DNA, 18 bp, Artificial Sequence
  AmNA[+23/+40]
  modified_base (1)..(1): c = AmNA_c
  modified_base (1)..(1): m5c
  modified_base (2)..(18): phosphorotioated
  modified_base (3)..(3): c = AmNA_c
  modified_base (3)..(3): m5c
  modified_base (5)..(5): c = AmNA_c
  modified_base (5)..(5): m5c
  modified_base (7)..(7): c = AmNA_c
  modified_base (7)..(7): m5c
  modified_base (9)..(9): a = AmNA_a
  modified_base (11)..(11): t = AmNA_t
  modified_base (13)..(13): a = AmNA_a
  modified_base (15)..(15): t = AmNA_t
  modified_base (17)..(17): t = AmNA_t
cacactctagtaaatatt

SEQ ID NO: 24 - DNA, 18 bp, Artificial Sequence
  AmNA[+27/+44]
  modified_base (1)..(1): a = AmNA_a
  modified_base (2)..(18): phosphorotioated
  modified_base (3)..(3): a = AmNA_a
  modified_base (5)..(5): c = AmNA_c
  modified_base (5)..(5): m5c
  modified_base (7)..(7): c = AmNA_c
  modified_base (7)..(7): m5c
  modified_base (9)..(9): c = AmNA_c
  modified_base (9)..(9): m5c
  modified_base (11)..(11): c = AmNA_c
  modified_base (11)..(11): m5c
  modified_base (13)..(13): a = AmNA_a
  modified_base (15)..(15): t = AmNA_t
  modified_base (17)..(17): a = AmNA_a
agatcacactctagtaaa

SEQ ID NO: 25 - DNA, 18 bp, Artificial Sequence
  AmNA[+31/+48]
  modified_base (1)..(1): a = AmNA_a
  modified_base (2)..(18): phosphorotioated
  modified_base (3)..(3): c = AmNA_c
  modified_base (3)..(3): m5c
  modified_base (5)..(5): a = AmNA_a
  modified_base (7)..(7): a = AmNA_a
  modified_base (9)..(9): c = AmNA_c
  modified_base (9)..(9): m5c
  modified_base (11)..(11): c = AmNA_c
  modified_base (11)..(11): m5c
  modified_base (13)..(13): c = AmNA_c
  modified_base (13)..(13): m5c
  modified_base (15)..(15): c = AmNA_c
  modified_base (15)..(15): m5c
  modified_base (17)..(17): a = AmNA_a
atctagatcacactctag

SEQ ID NO: 26 - DNA, 18 bp, Artificial Sequence
  AmNA[+35/-2(3')]
  modified_base (1)..(1): a = AmNA_a
  modified_base (2)..(18): phosphorotioated
  modified_base (3)..(3): c = AmNA_c
  modified_base (3)..(3): m3c
  modified_base (5)..(5): a = AmNA_a
  modified_base (7)..(7): c = AmNA_c
  modified_base (7)..(7): m3c
  modified_base (9)..(9): a = AmNA_a
  modified_base (11)..(11): a = AmNA_a
  modified_base (13)..(13): c = AmNA_c
  modified_base (13)..(13): m3c
  modified_base (15)..(15): c = AmNA_c
  modified_base (15)..(15): m3c
  modified_base (17)..(17): c = AmNA_c
acccatctagatcacact

SEQ ID NO: 27 - DNA, 18 bp, Artificial Sequence
  AmNA[+43/-10(3')]
  modified_base (1)..(1): g = AmNA_g
  modified_base (3)..(3): a = AmNA_a
  modified_base (5)..(5): a = AmNA_a
  modified_base (7)..(7): a = AmNA_a
  modified_base (9)..(9): a = AmNA_a
  modified_base (11)..(11): c = AmNA_c
  modified_base (11)..(11): m5c
  modified_base (13)..(13): a = AmNA_a
  modified_base (15)..(15): c = AmNA_c
  modified_base (15)..(15): m5c
  modified_base (17)..(17): a = AmNA_a
gaatacatacccatctag

SEQ ID NO: 28 - DNA, 18 bp, Artificial Sequence
  AmNA[-5(3')/-22(3')]
  modified_base (1)..(1): t = AmNA_t
  modified_base (2)..(18): phosphorotioated
  modified_base (3)..(3): c = AmNA_c
  modified_base (3)..(3): m5c
  modified_base (5)..(5): t = AmNA_t
  modified_base (7)..(7): c = AmNA_c
  modified_base (7)..(7): m5c
  modified_base (9)..(9): a = AmNA_a
  modified_base (11)..(11): c = AmNA_c
  modified_base (11)..(11): m5c
  modified_base (17)..(17): a = AmNA_a
tacattctacctgaatac

SEQ ID NO: 29 - DNA, 18 bp, Artificial Sequence
  AmNA[-17(3')/-34(3')]
  modified_base (1)..(1): g = AmNA_g
  modified_base (3)..(3): a = AmNA_a
  modified_base (5)..(5): a = AmNA_a
  modified_base (7)..(7): g = AmNA_g
  modified_base (9)..(9): g = AmNA_g
  modified_base (11)..(11): a = AmNA_a
  modified_base (13)..(13): t = AmNA_t
  modified_base (15)..(15): t = AmNA_t
  modified_base (15)..(15): c = AmNA_c
  modified_base (15)..(15): m5c
  modified_base (17)..(17): t = AmNA_t
gcataagagtaatacatt

SEQ ID NO: 30 - DNA, 21 bp, Artificial Sequence
  hSRRM4 For.Primer
tgacaaagacttgacaccacc

SEQ ID NO: 31 - DNA, 19 bp, Artificial Sequence
  hSRRM4 Rev.Primer
acctgcgtcgcttgtgttt

SEQ ID NO: 32 - DNA, 27 bp, Artificial Sequence
  TaqMan Probe
aggtcctcatcctatagcccatcgcct

SEQ ID NO: 33 - DNA, 21 bp, Artificial Sequence
  REST For.Primer
gaacgcccatataaatgtgaa

SEQ ID NO: 34 - DNA, 24 bp, Artificial Sequence
  REST Rev.Primer
tttgaagttgcttctatctgctgt

SEQ ID NO: 35 - DNA, 20 bp, Artificial Sequence
  beta-actin For.Primer
ggccgtcttcccctccatcg

SEQ ID NO: 36 - DNA, 22 bp, Artificial Sequence
  beta-actin Rev.Primer
ccagttggtgacgatgccgtgc

SEQ ID NO: 37 - DNA, 15 bp, Artificial Sequence
  AmNA_26
  modified_base (1)..(3): AmNA
  modified_base (2)..(15): phosphorotioated
  modified_base (13)..(14): AmNA
tgaacaaaataatac

SEQ ID NO: 38 - RNA, 26 nt, Homo sapiens
guaauauuuacuagagugugaucuag

SEQ ID NO: 39 - RNA, 24 nt, Homo sapiens
guaauauuuacuagagugugaucu

SEQ ID NO: 40 - DNA, 20 bp, Artificial Sequence
  [+23/+42]
atcacactctagtaaatatt

SEQ ID NO: 41 - DNA, 20 bp, Artificial Sequence
  [+21/+40]
cacactctagtaaatattac

SEQ ID NO: 42 - DNA, 16 bp, Artificial Sequence
  [+23/+38]
cactctagtaaatatt

SEQ ID NO: 43 - DNA, 16 bp, Artificial Sequence
  [+25/+40]
cacactctagtaaata

SEQ ID NO: 44 - DNA, 20 bp, Artificial Sequence
  [+27/+46]
ctagatcacactctagtaaa

SEQ ID NO: 45 - DNA, 20 bp, Artificial Sequence
  [+25/+44]
agatcacactctagtaaata

SEQ ID NO: 46 - DNA, 16 bp, Artificial Sequence
  [+27/+42]
atcacactctagtaaa

SEQ ID NO: 47 - DNA, 16 bp, Artificial Sequence
  [+29/+44]
agatcacactctagta

SEQ ID NO: 48 - DNA, 22 bp, Artificial Sequence
  [+23/+44]
agatcacactctagtaaatatt

SEQ ID NO: 49 - DNA, 18 bp, Artificial Sequence
  [+26/+43]
gatcacactctagtaaat

SEQ ID NO: 50 - RNA, 81 nt, Homo sapiens
uucuacuaugcauuccauuggaccagugggguauggauaccauuugguaauauuuacuagagugugaucuagauggguaug

SEQ ID NO: 51 - RNA, 135 nt, Homo sapiens
ucauaaaugucaauuuccguuuuucuacuaugcauuccauuggaccagugggguauggauaccauuugguaauauuuacuagagugugaucuagauggguauguauucagguagaauguauuacucuuaugccuu

SEQ ID NO: 52 - RNA, 48 nt, Homo sapiens
gauaccauuugguaauauuuacuagagugugaucuagauggguaugua

SEQ ID NO: 53 - DNA, 20 bp, Artificial Sequence
  AmNA[+23/+42]
  modified_base (1)..(1): a = AmNA_a
  modified_base (2)..(20): phosphorotioated
  modified_base (3)..(3): c = AmNA_c
  modified_base (3)..(3): m5c
  modified_base (5)..(5): c = AmNA_c
  modified_base (5)..(5): m5c
  modified_base (7)..(7): c = AmNA_c
  modified_base (7)..(7): m5c
  modified_base (9)..(9): c = AmNA_c
  modified_base (9)..(9): m5c
  modified_base (11)..(11): a = AmNA_a
  modified_base (13)..(13): t = AmNA_t
  modified_base (15)..(15): a = AmNA_a
  modified_base (17)..(17): t = AmNA_t
  modified_base (19)..(19): t = AmNA_t
atcacactctagtaaatatt

SEQ ID NO: 54 - DNA, 20 bp, Artificial Sequence
  AmNA[+21/+40]
  modified_base (1)..(1): c = AmNA_c
  modified_base (1)..(1): m5c
  modified_base (2)..(20): phosphorotioated
  modified_base (3)..(3): c = AmNA_c
  modified_base (3)..(3): m5c
  modified_base (5)..(5): c = AmNA_c
  modified_base (5)..(5): m5c
  modified_base (7)..(7): c = AmNA_c
  modified_base (7)..(7): m5c
  modified_base (9)..(9): a = AmNA_a
  modified_base (11)..(11): t = AmNA_t
  modified_base (13)..(13): a = AmNA_a
  modified_base (15)..(15): t = AmNA_t
  modified_base (17)..(17): t = AmNA_t
  modified_base (19)..(19): a = AmNA_a
cacactctagtaaatattac

SEQ ID NO: 55 - DNA, 16 bp, Artificial Sequence
  AmNA[+23/+38]
  modified_base (1)..(1): c = AmNA_c
  modified_base (1)..(1): m5c
  modified_base (2)..(16): phosphorotioated
  modified_base (3)..(3): c = AmNA_c
  modified_base (3)..(3): m5c
  modified_base (5)..(5): c = AmNA_c
  modified_base (5)..(5): m5c
  modified_base (7)..(7): a = AmNA_a
  modified_base (9)..(9): t = AmNA_t
  modified_base (11)..(11): a = AmNA_a
  modified_base (13)..(13): t = AmNA_t
  modified_base (15)..(15): t = AmNA_t
cactctagtaaatatt

SEQ ID NO: 56 - DNA, 16 bp, Artificial Sequence
  AmNA[+25/+40]
  modified_base (1)..(1): c = AmNA_c
  modified_base (1)..(1): m5c
  modified_base (2)..(16): phosphorotioated
  modified_base (3)..(3): c = AmNA_c
  modified_base (3)..(3): m5c
  modified_base (5)..(5): c = AmNA_c
  modified_base (5)..(5): m5c
  modified_base (7)..(7): c = AmNA_c
  modified_base (7)..(7): m5c
  modified_base (9)..(9): a = AmNA_a
  modified_base (11)..(11): t = AmNA_t
  modified_base (13)..(13): a = AmNA_a
  modified_base (15)..(15): t = AmNA_t
cacactctagtaaata

SEQ ID NO: 57 - DNA, 20 bp, Artificial Sequence
  AmNA[+27/+46]
  modified_base (1)..(1): c = AmNA_c
  modified_base (1)..(1): m5c
  modified_base (2)..(20): phosphorotioated
  modified_base (3)..(3): a = AmNA_a
  modified_base (5)..(5): a = AmNA_a
  modified_base (7)..(7): c = AmNA_c
  modified_base (7)..(7): m5c
  modified_base (9)..(9): c = AmNA_c
  modified_base (9)..(9): m5c
  modified_base (11)..(11): c = AmNA_c
  modified_base (11)..(11): m5c
  modified_base (13)..(13): c = AmNA_c
  modified_base (13)..(13): m5c
  modified_base (15)..(15): a = AmNA_a
  modified_base (17)..(17): t = AmNA_t
  modified_base (19)..(19): a = AmNA_a
ctagatcacactctagtaaa

SEQ ID NO: 58 - DNA, 20 bp, Artificial Sequence
  AmNA[+25/+44]
  modified_base (1)..(1): a = AmNA_a
  modified_base (2)..(20): phosphorotioated
  modified_base (3)..(3): a = AmNA_a
  modified_base (5)..(5): c = AmNA_c
  modified_base (5)..(5): m5c
  modified_base (7)..(7): c = AmNA_c
  modified_base (7)..(7): m5c
  modified_base (9)..(9): c = AmNA_c
  modified_base (9)..(9): m5c
  modified_base (11)..(11): c = AmNA_c
  modified_base (11)..(11): m5c
  modified_base (13)..(13): a = AmNA_a
  modified_base (15)..(15): t = AmNA_t
  modified_base (17)..(17): a = AmNA_a
  modified_base (19)..(19): t = AmNA_t
agatcacactctagtaaata

SEQ ID NO: 59 - DNA, 16 bp, Artificial Sequence
  AmNA[+27/+42]
  modified_base (1)..(1): a = AmNA_a
  modified_base (2)..(16): phosphorotioated
  modified_base (3)..(3): c = AmNA_c
  modified_base (3)..(3): m5c
  modified_base (5)..(5): c = AmNA_c
  modified_base (5)..(5): m5c
  modified_base (7)..(7): c = AmNA_c
  modified_base (7)..(7): m5c
  modified_base (9)..(9): c = AmNA_c
  modified_base (9)..(9): m5c
  modified_base (11)..(11): a = AmNA_a
  modified_base (13)..(13): t = AmNA_t
  modified_base (15)..(15): a = AmNA_a
atcacactctagtaaa

SEQ ID NO: 60 - DNA, 16 bp, Artificial Sequence
  AmNA[+29/+44]
  modified_base (1)..(1): a = AmNA_a
  modified_base (2)..(16): phosphorotioated
  modified_base (3)..(3): a = AmNA_a
  modified_base (5)..(5): c = AmNA_c
  modified_base (5)..(5): m5c
  modified_base (7)..(7): c = AmNA_c
  modified_base (7)..(7): m5c
  modified_base (9)..(9): c = AmNA_c
  modified_base (9)..(9): m5c
  modified_base (11)..(11): c = AmNA_c
  modified_base (11)..(11): m5c
  modified_base (13)..(13): a = AmNA_a
  modified_base (15)..(15): t = AmNA_t
agatcacactctagta

SEQ ID NO: 61 - DNA, 22 bp, Artificial Sequence
  AmNA[+23/+44]
  modified_base (1)..(1): a = AmNA_a
  modified_base (2)..(22): phosphorotioated
  modified_base (3)..(3): a = AmNA_a
  modified_base (5)..(5): c = AmNA_c
  modified_base (5)..(5): m5c
  modified_base (7)..(7): c = AmNA_c
  modified_base (7)..(7): m5c
  modified_base (9)..(9): c = AmNA_c
  modified_base (9)..(9): m5c
  modified_base (11)..(11): c = AmNA_c
  modified_base (11)..(11): m5c
  modified_base (13)..(13): a = AmNA_a
  modified_base (15)..(15): t = AmNA_t
  modified_base (17)..(17): a = AmNA_a
  modified_base (19)..(19): t = AmNA_t
  modified_base (21)..(21): t = AmNA_t
agatcacactctagtaaatatt

SEQ ID NO: 62 - DNA, 18 bp, Artificial Sequence
  AmNA[+26/+43]
  modified_base (1)..(1): g = AmNA_g
  modified_base (2)..(18): phosphorotioated
  modified_base (3)..(3): t = AmNA_t
  modified_base (5)..(5): a = AmNA_a
  modified_base (7)..(7): a = AmNA_a
  modified_base (9)..(9): t = AmNA_t
  modified_base (11)..(11): t = AmNA_t
  modified_base (13)..(13): g = AmNA_g
  modified_base (15)..(15): a = AmNA_a
  modified_base (17)..(17): a = AmNA_a
gatcacactctagtaaat

SEQ ID NO: 63 - DNA, 18 bp, Artificial Sequence
  AmNA[+27/+44]_1/3
  modified_base (1)..(1): a = AmNA_a
  modified_base (2)..(18): phosphorotioated
  modified_base (4)..(4): t = AmNA_t
  modified_base (7)..(7): c = AmNA_c
  modified_base (7)..(7): m5c
  modified_base (10)..(10): t = AmNA_t
  modified_base (13)..(13): a = AmNA_a
  modified_base (16)..(16): a = AmNA_a
agatcacactctagtaaa

SEQ ID NO: 64 - DNA, 18 bp, Artificial Sequence
  NC1
  modified_base (1)..(1): c = AmNA_c
  modified_base (1)..(1): m5c
  modified_base (2)..(18): phosphorotioated
  modified_base (3)..(3): c = AmNA_c
  modified_base (3)..(3): m5c
  modified_base (5)..(5): t = AmNA_t
  modified_base (7)..(7): t = AmNA_t
  modified_base (9)..(9): g = AmNA_g
  modified_base (11)..(11): a = AmNA_a
  modified_base (13)..(13): a = AmNA_a
  modified_base (15)..(15): a = AmNA_a
  modified_base (17)..(17): t = AmNA_t
cacctatcgtaaacactc

SEQ ID NO: 65 - DNA, 18 bp, Artificial Sequence
  NC2
  modified_base (1)..(1): c = AmNA_c
  modified_base (1)..(1): m5c
  modified_base (2)..(18): phosphorotioated
  modified_base (3)..(3): a = AmNA_a
  modified_base (5)..(5): c = AmNA_c
  modified_base (5)..(5): m5c
  modified_base (7)..(7): a = AmNA_a
  modified_base (9)..(9): c = AmNA_c
  modified_base (9)..(9): m5c
  modified_base (11)..(11): a = AmNA_a
  modified_base (13)..(13): a = AmNA_a
  modified_base (15)..(15): c = AmNA_c
  modified_base (15)..(15): m5c
  modified_base (17)..(17): c = AmNA_c
  modified_base (17)..(17): m5c
ccacctagcaatatcact

SEQ ID NO: 66 - DNA, 18 bp, Artificial Sequence
  NC3
  modified_base (1)..(1): c = AmNA_c
  modified_base (1)..(1): m5c
  modified_base (2)..(18): phosphorotioated
  modified_base (3)..(3): c = AmNA_c
  modified_base (3)..(3): m5c
  modified_base (5)..(5): a = AmNA_a
  modified_base (7)..(7): a = AmNA_a
  modified_base (9)..(9): c = AmNA_c
  modified_base (9)..(9): m5c
  modified_base (11)..(11): a = AmNA_a
  modified_base (13)..(13): c = AmNA_c
  modified_base (13)..(13): m5c
  modified_base (15)..(15): c = AmNA_c
  modified_base (15)..(15): m5c
  modified_base (17)..(17): a = AmNA_a
cgccacaactatcactat

SEQ ID NO: 67 - DNA, 18 bp, Artificial Sequence
  NC4
  modified_base (1)..(1): c = AmNA_c
  modified_base (1)..(1): m5c
  modified_base (2)..(18): phosphorotioated
  modified_base (3)..(3): c = AmNA_c
  modified_base (3)..(3): m5c
  modified_base (5)..(5): a = AmNA_a
  modified_base (7)..(7): a = AmNA_a
  modified_base (9)..(9): c = AmNA_c
  modified_base (9)..(9): m5c
  modified_base (11)..(11): a = AmNA_a
  modified_base (13)..(13): c = AmNA_c
  modified_base (13)..(13): m5c
  modified_base (15)..(15): c = AmNA_c
  modified_base (15)..(15): m5c
  modified_base (17)..(17): a = AmNA_a
cacgaaatctatccccat